European Patent Application EP 4 212 634 A1, published July 19, 2023. Title: COMPOSITIONS AND METHODS FOR DETECTION OF VIRAL PATHOGENS IN SAMPLES. Applicant: Gen-Probe Incorporated. Application EP. The sequence listing filed with the application follows.

SEQUENCE LISTING (119 sequences)

SEQ ID NO: 1 - DNA, 18 bp, synthetic construct
  misc_feature 1..18: note = Synthetic Oligonucleotide
  source 1..18: mol_type = other DNA
gatcttgaggctctcatg

SEQ ID NO: 2 - DNA, 20 bp, synthetic construct
  misc_feature 1..20: note = Synthetic Oligonucleotide
  source 1..20: mol_type = other DNA
ataacrttccatggrgccaa

SEQ ID NO: 3 - DNA, 20 bp, synthetic construct
  misc_feature 1..20: note = Synthetic Oligonucleotide
  source 1..20: mol_type = other DNA
ataacrttccatggggccaa

SEQ ID NO: 4 - DNA, 19 bp, synthetic construct
  misc_feature 1..19: note = Synthetic Oligonucleotide
  source 1..19: mol_type = other DNA
ataacgttccatggrgcca

SEQ ID NO: 5 - DNA, 20 bp, synthetic construct
  misc_feature 1..20: note = Synthetic Oligonucleotide
  source 1..20: mol_type = other DNA
ataacgttccatggggccaa

SEQ ID NO: 6 - DNA, 20 bp, synthetic construct
  misc_feature 1..20: note = Synthetic Oligonucleotide
  source 1..20: mol_type = other DNA
cccttagtcagaggtgacag

SEQ ID NO: 7 - DNA, 27 bp, synthetic construct
  misc_feature 1..27: note = Synthetic Oligonucleotide
  source 1..27: mol_type = other DNA
tcaggccccctcaaagccgagatcgcc

SEQ ID NO: 8 - DNA, 26 bp, synthetic construct
  misc_feature 1..26: note = Synthetic Oligonucleotide
  source 1..26: mol_type = other DNA
tcaggccccctcaaagccgaratcgc

SEQ ID NO: 9 - DNA, 26 bp, synthetic construct
  misc_feature 1..26: note = Synthetic Oligonucleotide
  source 1..26: mol_type = other DNA
tcaggccccctcaaagccgagatcgc

SEQ ID NO: 10 - DNA, 26 bp, synthetic construct
  misc_feature 1..26: note = Synthetic Oligonucleotide
  source 1..26: mol_type = other DNA
  modified_base 5..6: mod_base = OTHER; note = uracil
  modified_base 12..14: mod_base = OTHER; note = uracil
  modified_base 24: mod_base = OTHER; note = uracil
gcgatttcggctttgagggggcctga

SEQ ID NO: 11 - DNA, 26 bp, synthetic construct
  misc_feature 1..26: note = Synthetic Oligonucleotide
  source 1..26: mol_type = other DNA
  modified_base 5: mod_base = OTHER; note = uracil
  modified_base 12..14: mod_base = OTHER; note = uracil
  modified_base 24: mod_base = OTHER; note = uracil
gcgatctcggctttgagggggcctga

SEQ ID NO: 12 - DNA, 27 bp, synthetic construct
  misc_feature 1..27: note = Synthetic Oligonucleotide
  source 1..27: mol_type = other DNA
  modified_base 6: mod_base = OTHER; note = uracil
agccattccatgagagcctcaagatcc

SEQ ID NO: 13 - DNA, 26 bp, synthetic construct
  misc_feature 1..26: note = Synthetic Oligonucleotide
  source 1..26: mol_type = other DNA
agccaytccatragagcctcaagatc

SEQ ID NO: 14 - DNA, 26 bp, synthetic construct
  misc_feature 1..26: note = Synthetic Oligonucleotide
  source 1..26: mol_type = other DNA
  modified_base 6: mod_base = OTHER; note = uracil
agccattccatgagagcctcaagatc

SEQ ID NO: 15 - DNA, 26 bp, synthetic construct
  misc_feature 1..26: note = Synthetic Oligonucleotide
  source 1..26: mol_type = other DNA
  modified_base 3: mod_base = OTHER; note = uracil
  modified_base 5..6: mod_base = OTHER; note = uracil
  modified_base 12: mod_base = OTHER; note = uracil
  modified_base 14: mod_base = OTHER; note = uracil
  modified_base 17: mod_base = OTHER; note = uracil
  modified_base 22: mod_base = OTHER; note = uracil
  modified_base 26: mod_base = OTHER; note = uracil
gatcttgaggctctcatggagtggct

SEQ ID NO: 16 - DNA, 26 bp, synthetic construct
  misc_feature 1..26: note = Synthetic Oligonucleotide
  source 1..26: mol_type = other DNA
  modified_base 3: mod_base = OTHER; note = uracil
  modified_base 5..6: mod_base = OTHER; note = uracil
  modified_base 12: mod_base = OTHER; note = uracil
  modified_base 14: mod_base = OTHER; note = uracil
  modified_base 17: mod_base = OTHER; note = uracil
  modified_base 22: mod_base = OTHER; note = uracil
  modified_base 26: mod_base = OTHER; note = uracil
gatcttgaggctctcatggaatggct

SEQ ID NO: 17 - DNA, 26 bp, synthetic construct
  misc_feature 1..26: note = Synthetic Oligonucleotide
  source 1..26: mol_type = other DNA
  modified_base 3: mod_base = OTHER; note = uracil
  modified_base 5..6: mod_base = OTHER; note = uracil
  modified_base 12: mod_base = OTHER; note = uracil
  modified_base 14..15: mod_base = OTHER; note = uracil
  modified_base 17: mod_base = OTHER; note = uracil
  modified_base 22: mod_base = OTHER; note = uracil
  modified_base 26: mod_base = OTHER; note = uracil
gatcttgaggctcttatggaatggct

SEQ ID NO: 18 - DNA, 24 bp, synthetic construct
  misc_feature 1..24: note = Synthetic Oligonucleotide
  source 1..24: mol_type = other DNA
  modified_base 20: mod_base = OTHER; note = uracil
ctggtgcacttgccagttgtatgc

SEQ ID NO: 19 - DNA, 23 bp, synthetic construct
  misc_feature 1..23: note = Synthetic Oligonucleotide
  source 1..23: mol_type = other DNA
ctggtgcacttgccagttcyatg

SEQ ID NO: 20 - DNA, 23 bp, synthetic construct
  misc_feature 1..23: note = Synthetic Oligonucleotide
  source 1..23: mol_type = other DNA
  modified_base 20: mod_base = OTHER; note = uracil
ctggtgcacttgccagttctatg

SEQ ID NO: 21 - DNA, 23 bp, synthetic construct
  misc_feature 1..23: note = Synthetic Oligonucleotide
  source 1..23: mol_type = other DNA
  modified_base 3: mod_base = OTHER; note = uracil
  modified_base 9: mod_base = OTHER; note = uracil
  modified_base 16: mod_base = OTHER; note = uracil
catagaactggcaagtgcaccag

SEQ ID NO: 22 - DNA, 23 bp, synthetic construct
  misc_feature 1..23: note = Synthetic Oligonucleotide
  source 1..23: mol_type = other DNA
  modified_base 3: mod_base = OTHER; note = uracil
  modified_base 9: mod_base = OTHER; note = uracil
  modified_base 16: mod_base = OTHER; note = uracil
catggaactggcaagtgcaccag

SEQ ID NO: 23 - DNA, 22 bp, synthetic construct
  misc_feature 1..22: note = Synthetic Oligonucleotide
  source 1..22: mol_type = other DNA
cttctaaccgaggtcgaaacgt

SEQ ID NO: 24 - DNA, 20 bp, synthetic construct
  misc_feature 1..20: note = Synthetic Oligonucleotide
  source 1..20: mol_type = other DNA
ataacgttccatggggccaa

SEQ ID NO: 25 - DNA, 19 bp, synthetic construct
  misc_feature 1..19: note = Synthetic Oligonucleotide
  source 1..19: mol_type = other DNA
cccttagtcagaggtgaca

SEQ ID NO: 26 - DNA, 20 bp, synthetic construct
  misc_feature 1..20: note = Synthetic Oligonucleotide
  source 1..20: mol_type = other DNA
cccattctgttgtatatgag

SEQ ID NO: 27 - DNA, 20 bp, synthetic construct
  misc_feature 1..20: note = Synthetic Oligonucleotide
  source 1..20: mol_type = other DNA
cccatcctgttgtatatgag

SEQ ID NO: 28 - DNA, 18 bp, synthetic construct
  misc_feature 1..18: note = Synthetic Oligonucleotide
  source 1..18: mol_type = other DNA
ggtgagcgtgaacacaaa

SEQ ID NO: 29 - DNA, 22 bp, synthetic construct
  misc_feature 1..22: note = Synthetic Oligonucleotide
  source 1..22: mol_type = other DNA
agtggaggatgaagaagatggc

SEQ ID NO: 30 - DNA, 33 bp, synthetic construct
  misc_feature 1..33: note = Synthetic Oligonucleotide
  source 1..33: mol_type = other DNA
gcctgctttgccttctccatcttctgtgcaggc

SEQ ID NO: 31 - DNA, 26 bp, synthetic construct
  misc_feature 1..26: note = Synthetic Oligonucleotide
  source 1..26: mol_type = other DNA
gcctgctttgccttctccatcttctg

SEQ ID NO: 32 - DNA, 34 bp, synthetic construct
  misc_feature 1..34: note = Synthetic Oligonucleotide
  source 1..34: mol_type = other DNA
gcctgctttgccttctccatcttctgtagcaggc

SEQ ID NO: 33 - DNA, 27 bp, synthetic construct
  misc_feature 1..27: note = Synthetic Oligonucleotide
  source 1..27: mol_type = other DNA
gcctgctttgccttctccatcttctgt

SEQ ID NO: 34 - DNA, 38 bp, synthetic construct
  misc_feature 1..38: note = Synthetic Oligonucleotide
  source 1..38: mol_type = other DNA
gcgctagttctgctttgccttctccatcttcctagcgc

SEQ ID NO: 35 - DNA, 31 bp, synthetic construct
  misc_feature 1..31: note = Synthetic Oligonucleotide
  source 1..31: mol_type = other DNA
gcgctagttctgctttgccttctccatcttc

SEQ ID NO: 36 - DNA, 38 bp, synthetic construct; identical to SEQ ID NO: 34
  misc_feature 1..38: note = Synthetic Oligonucleotide
  source 1..38: mol_type = other DNA

SEQ ID NO: 37 - DNA, 31 bp, synthetic construct; identical to SEQ ID NO: 35
  misc_feature 1..31: note = Synthetic Oligonucleotide
  source 1..31: mol_type = other DNA

SEQ ID NO: 38 - DNA, 38 bp, synthetic construct; identical to SEQ ID NO: 34
  misc_feature 1..38: note = Synthetic Oligonucleotide
  source 1..38: mol_type = other DNA

SEQ ID NO: 39 - DNA, 31 bp, synthetic construct; identical to SEQ ID NO: 35
  misc_feature 1..31: note = Synthetic Oligonucleotide
  source 1..31: mol_type = other DNA

SEQ ID NO: 40 - DNA, 34 bp, synthetic construct
  misc_feature 1..34: note = Synthetic Oligonucleotide
  source 1..34: mol_type = other DNA
gctgctagttctgctttgccttctccatcgcagc

SEQ ID NO: 41 - DNA, 29 bp, synthetic construct
  misc_feature 1..29: note = Synthetic Oligonucleotide
  source 1..29: mol_type = other DNA
gctgctagttctgctttgccttctccatc

SEQ ID NO: 42 - DNA, 36 bp, synthetic construct
  misc_feature 1..36: note = Synthetic Oligonucleotide
  source 1..36: mol_type = other DNA
gcctgctagttctgctttgccttctccatcgcaggc

SEQ ID NO: 43 - DNA, 30 bp, synthetic construct
  misc_feature 1..30: note = Synthetic Oligonucleotide
  source 1..30: mol_type = other DNA
gcctgctagttctgctttgccttctccatc

SEQ ID NO: 44 - DNA, 36 bp, synthetic construct; identical to SEQ ID NO: 42
  misc_feature 1..36: note = Synthetic Oligonucleotide
  source 1..36: mol_type = other DNA

SEQ ID NO: 45 - DNA, 30 bp, synthetic construct; identical to SEQ ID NO: 43
  misc_feature 1..30: note = Synthetic Oligonucleotide
  source 1..30: mol_type = other DNA

SEQ ID NO: 46 - DNA, 37 bp, synthetic construct
  misc_feature 1..37: note = Synthetic Oligonucleotide
  source 1..37: mol_type = other DNA
gcctgctagttctgctttgccttctccatcagcaggc

SEQ ID NO: 47 - DNA, 30 bp, synthetic construct; identical to SEQ ID NO: 43
  misc_feature 1..30: note = Synthetic Oligonucleotide
  source 1..30: mol_type = other DNA

SEQ ID NO: 48 - DNA, 37 bp, synthetic construct; identical to SEQ ID NO: 46
  misc_feature 1..37: note = Synthetic Oligonucleotide
  source 1..37: mol_type = other DNA

SEQ ID NO: 49 - DNA, 30 bp, synthetic construct; identical to SEQ ID NO: 43
  misc_feature 1..30: note = Synthetic Oligonucleotide
  source 1..30: mol_type = other DNA

SEQ ID NO: 50 - DNA, 37 bp, synthetic construct; identical to SEQ ID NO: 46
  misc_feature 1..37: note = Synthetic Oligonucleotide
  source 1..37: mol_type = other DNA

SEQ ID NO: 51 - DNA, 30 bp, synthetic construct; identical to SEQ ID NO: 43
  misc_feature 1..30: note = Synthetic Oligonucleotide
  source 1..30: mol_type = other DNA

SEQ ID NO: 52 - DNA, 38 bp, synthetic construct
  misc_feature 1..38: note = Synthetic Oligonucleotide
  source 1..38: mol_type = other DNA
gcctgctagttctgctttgccttctccatctagcaggc

SEQ ID NO: 53 - DNA, 30 bp, synthetic construct; identical to SEQ ID NO: 43
  misc_feature 1..30: note = Synthetic Oligonucleotide
  source 1..30: mol_type = other DNA

SEQ ID NO: 54 - DNA, 34 bp, synthetic construct
  misc_feature 1..34: note = Synthetic Oligonucleotide
  source 1..34: mol_type = other DNA
  modified_base 21: mod_base = OTHER; note = uracil
gcggagaaggcaaagcagaattagcagtctccgc

SEQ ID NO: 55 - DNA, 27 bp, synthetic construct
  misc_feature 1..27: note = Synthetic Oligonucleotide
  source 1..27: mol_type = other DNA
  modified_base 21: mod_base = OTHER; note = uracil
gcggagaaggcaaagcagaattagcag

SEQ ID NO: 56 - DNA, 34 bp, synthetic construct; identical to SEQ ID NO: 54
  misc_feature 1..34: note = Synthetic Oligonucleotide
  source 1..34: mol_type = other DNA
  modified_base 21: mod_base = OTHER; note = uracil

SEQ ID NO: 57 - DNA, 27 bp, synthetic construct
  misc_feature 1..27: note = Synthetic Oligonucleotide
  source 1..27: mol_type = other DNA
  modified_base 21: mod_base = OTHER; note = uracil
gcggagaaggcaaagcagaattagcag

SEQ ID NO: 58 - DNA, 20 bp, synthetic construct
  misc_feature 1..20: note = Synthetic Oligonucleotide
  source 1..20: mol_type = other DNA
tctttcccaccraaccaaca

SEQ ID NO: 59 - DNA, 29 bp, synthetic construct
  misc_feature 1..29: note = Synthetic Oligonucleotide
  source 1..29: mol_type = other DNA
ctagttctgctttgccttctccatcttct

SEQ ID NO: 60 - DNA, 24 bp, synthetic construct
  misc_feature 1..24: note = Synthetic Oligonucleotide
  source 1..24: mol_type = other DNA
aagactcccaccgcagtttcagct

SEQ ID NO: 61 - DNA, 24 bp, synthetic construct
  misc_feature 1..24: note = Synthetic Oligonucleotide
  source 1..24: mol_type = other DNA
aagactcccaccgcagtttcagct

SEQ ID NO: 62 - DNA, 24 bp, synthetic construct
  misc_feature 1..24: note = Synthetic Oligonucleotide
  source 1..24: mol_type = other DNA
aagactcccaccgcagtttcagct

SEQ ID NO: 63 - DNA, 29 bp, synthetic construct
  misc_feature 1..29: note = Synthetic Oligonucleotide
  source 1..29: mol_type = other DNA
ctarttctgctttgccttctccatcttct

SEQ ID NO: 64 - DNA, 29 bp, synthetic construct
  misc_feature 1..29: note = Synthetic Oligonucleotide
  source 1..29: mol_type = other DNA
ctagttctgctttgccttctccatcttct

SEQ ID NO: 65 - DNA, 29 bp, synthetic construct
  misc_feature 1..29: note = Synthetic Oligonucleotide
  source 1..29: mol_type = other DNA
  modified_base 7: mod_base = OTHER; note = uracil
  modified_base 26..27: mod_base = OTHER; note = uracil
agaagatggagaaggcaaagcagaattag

SEQ ID NO: 66 - DNA, 29 bp, synthetic construct
  misc_feature 1..29: note = Synthetic Oligonucleotide
  source 1..29: mol_type = other DNA
  modified_base 7: mod_base = OTHER; note = uracil
  modified_base 27: mod_base = OTHER; note = uracil
agaagatggagaaggcaaagcagaactag

SEQ ID NO: 67 - DNA, 23 bp, synthetic construct
  misc_feature 1..23: note = Synthetic Oligonucleotide
  source 1..23: mol_type = other DNA
gagacacaattgcctacctgctt

SEQ ID NO: 68 - DNA, 26 bp, synthetic construct
  misc_feature 1..26: note = Synthetic Oligonucleotide
  source 1..26: mol_type = other DNA
  modified_base 15: mod_base = OTHER; note = uracil
gagtctaggtcaaattctttcccacc

SEQ ID NO: 69 - DNA, 21 bp, synthetic construct
  misc_feature 1..21: note = Synthetic Oligonucleotide
  source 1..21: mol_type = other DNA
ggtgctcttgaccaaattggg

SEQ ID NO: 70 - DNA, 22 bp, synthetic construct
  misc_feature 1..22: note = Synthetic Oligonucleotide
  source 1..22: mol_type = other DNA
ctttcccaccraaccaacagtg

SEQ ID NO: 71 - DNA, 29 bp, synthetic construct
  misc_feature 1..29: note = Synthetic Oligonucleotide
  source 1..29: mol_type = other DNA
ttagtcatyacagtgactgacaacaaagg

SEQ ID NO: 72 - DNA, 23 bp, synthetic construct
  misc_feature 1..23: note = Synthetic Oligonucleotide
  source 1..23: mol_type = other DNA
aggtaagctccwagatctactat

SEQ ID NO: 73 - DNA, 23 bp, synthetic construct
  misc_feature 1..23: note = Synthetic Oligonucleotide
  source 1..23: mol_type = other DNA
aggtaagctccwagatctactat

SEQ ID NO: 74 - DNA, 23 bp, synthetic construct
  misc_feature 1..23: note = Synthetic Oligonucleotide
  source 1..23: mol_type = other DNA
aggtaagctcctagatctactat

SEQ ID NO: 75 - DNA, 32 bp, synthetic construct
  misc_feature 1..32: note = Synthetic Oligonucleotide
  source 1..32: mol_type = other DNA
  modified_base 9: mod_base = OTHER; note = uracil
ttagtcattacagtgactgacaacaaaggagc

SEQ ID NO: 76 - DNA, 21 bp, synthetic construct
  misc_feature 1..21: note = Synthetic Oligonucleotide
  source 1..21: mol_type = other DNA
tagaccatgtgaattccctgc

SEQ ID NO: 77 - DNA, 29 bp, synthetic construct
  misc_feature 1..29: note = Synthetic Oligonucleotide
  source 1..29: mol_type = other DNA
ttagtcatyacagtgactgacaacaaagg

SEQ ID NO: 78 - DNA, 29 bp, synthetic construct
  misc_feature 1..29: note = Synthetic Oligonucleotide
  source 1..29: mol_type = other DNA
  modified_base 9: mod_base = OTHER; note = uracil
ttagtcattacagtgactgacaacaaagg

SEQ ID NO: 79 - DNA, 26 bp, synthetic construct
  misc_feature 1..26: note = Synthetic Oligonucleotide
  source 1..26: mol_type = other DNA
acaaatgcaaaaatcataccttactc

SEQ ID NO: 80 - DNA, 36 bp, synthetic construct
  misc_feature 1..36: note = Synthetic Oligonucleotide
  source 1..36: mol_type = other DNA
cgtggctttatgtatttgaatgctcctttggccacg

SEQ ID NO: 81 - DNA, 30 bp, synthetic construct
  misc_feature 1..30: note = Synthetic Oligonucleotide
  source 1..30: mol_type = other DNA
cgtggctttatgtatttgaatgctcctttg

SEQ ID NO: 82 - DNA, 36 bp, synthetic construct; identical to SEQ ID NO: 80
  misc_feature 1..36: note = Synthetic Oligonucleotide
  source 1..36: mol_type = other DNA

SEQ ID NO: 83 - DNA, 30 bp, synthetic construct; identical to SEQ ID NO: 81
  misc_feature 1..30: note = Synthetic Oligonucleotide
  source 1..30: mol_type = other DNA

SEQ ID NO: 84 - DNA, 38 bp, synthetic construct
  misc_feature 1..38: note = Synthetic Oligonucleotide
  source 1..38: mol_type = other DNA
cggtggctttatgtatttgaatgctcctttggccaccg

SEQ ID NO: 85 - DNA, 31 bp, synthetic construct
  misc_feature 1..31: note = Synthetic Oligonucleotide
  source 1..31: mol_type = other DNA
cggtggctttatgtatttgaatgctcctttg

SEQ ID NO: 86 - DNA, 39 bp, synthetic construct
  misc_feature 1..39: note = Synthetic Oligonucleotide
  source 1..39: mol_type = other DNA
cggtggctttatgtatttgaatgctcctttgagccaccg

SEQ ID NO: 87 - DNA, 31 bp, synthetic construct; identical to SEQ ID NO: 85
  misc_feature 1..31: note = Synthetic Oligonucleotide
  source 1..31: mol_type = other DNA

SEQ ID NO: 88 - DNA, 26 bp, synthetic construct
  misc_feature 1..26: note = Synthetic Oligonucleotide
  source 1..26: mol_type = other DNA
acaaatgcaaaaatcataccttactc

SEQ ID NO: 89 - DNA, 29 bp, synthetic construct
  misc_feature 1..29: note = Synthetic Oligonucleotide
  source 1..29: mol_type = other DNA
ttagtcattacagtgactgacaacaaagg

SEQ ID NO: 90 - DNA, 29 bp, synthetic construct
  misc_feature 1..29: note = Synthetic Oligonucleotide
  source 1..29: mol_type = other DNA
ttagtcatyacagtgactgacaacaaagg

SEQ ID NO: 91 - DNA, 29 bp, synthetic construct
  misc_feature 1..29: note = Synthetic Oligonucleotide
  source 1..29: mol_type = other DNA
  modified_base 9: mod_base = OTHER; note = uracil
ttagtcattacagtgactgacaacaaagg

SEQ ID NO: 92 - DNA, 23 bp, synthetic construct
  misc_feature 1..23: note = Synthetic Oligonucleotide
  source 1..23: mol_type = other DNA
aggtaagctccgagatctactat

SEQ ID NO: 93 - DNA, 25 bp, synthetic construct
  misc_feature 1..25: note = Synthetic Oligonucleotide
  source 1..25: mol_type = other DNA
ctaggtaagctccaagatctactat

SEQ ID NO: 94 - DNA, 25 bp, synthetic construct
  misc_feature 1..25: note = Synthetic Oligonucleotide
  source 1..25: mol_type = other DNA
ctaggtaagctccaagatctactat

SEQ ID NO: 95 - DNA, 25 bp, synthetic construct
  misc_feature 1..25: note = Synthetic Oligonucleotide
  source 1..25: mol_type = other DNA
ctaggtaagctcctagatctactat

SEQ ID NO: 96 - DNA, 25 bp, synthetic construct
  misc_feature 1..25: note = Synthetic Oligonucleotide
  source 1..25: mol_type = other DNA
ctaggtaagctcctagatctactat

SEQ ID NO: 97 - DNA, 29 bp, synthetic construct
  misc_feature 1..29: note = Synthetic Oligonucleotide
  source 1..29: mol_type = other DNA
  modified_base 3..5: mod_base = OTHER; note = uracil
  modified_base 7..8: mod_base = OTHER; note = uracil
  modified_base 10: mod_base = OTHER; note = uracil
  modified_base 14: mod_base = OTHER; note = uracil
  modified_base 18: mod_base = OTHER; note = uracil
  modified_base 20: mod_base = OTHER; note = uracil
  modified_base 23: mod_base = OTHER; note = uracil
  modified_base 27: mod_base = OTHER; note = uracil
cctttgttgtcagtcactgtgatgactaa

SEQ ID NO: 98 - DNA, 29 bp, synthetic construct
  misc_feature 1..29: note = Synthetic Oligonucleotide
  source 1..29: mol_type = other DNA
  modified_base 3..5: mod_base = OTHER; note = uracil
  modified_base 7..8: mod_base = OTHER; note = uracil
  modified_base 10: mod_base = OTHER; note = uracil
  modified_base 14: mod_base = OTHER; note = uracil
  modified_base 18: mod_base = OTHER; note = uracil
  modified_base 20: mod_base = OTHER; note = uracil
  modified_base 23: mod_base = OTHER; note = uracil
  modified_base 27: mod_base = OTHER; note = uracil
cctttgttgtcagtcactgtaatgactaa

SEQ ID NO: 99 - DNA, 21 bp, synthetic construct
  misc_feature 1..21: note = Synthetic Oligonucleotide
  source 1..21: mol_type = other DNA
tgaagttgatgaacaaagtgg

SEQ ID NO: 100 - DNA, 23 bp, synthetic construct
  misc_feature 1..23: note = Synthetic Oligonucleotide
  source 1..23: mol_type = other DNA
gatgatgatccygcatcactaac

SEQ ID NO: 101 - DNA, 23 bp, synthetic construct
  misc_feature 1..23: note = Synthetic Oligonucleotide
  source 1..23: mol_type = other DNA
  modified_base 12: mod_base = OTHER; note = uracil
gatgatgatcctgcatcactaac

SEQ ID NO: 102 - DNA, 26 bp, synthetic construct
  misc_feature 1..26: note = Synthetic Oligonucleotide
  source 1..26: mol_type = other DNA
atgggtgcctatgttccagtcatctg

SEQ ID NO: 103 - DNA, 21 bp, synthetic construct
  misc_feature 1..21: note = Synthetic Oligonucleotide
  source 1..21: mol_type = other DNA
caccagccctcaataccaccc

SEQ ID NO: 104 - DNA, 19 bp, synthetic construct
  misc_feature 1..19: note = Synthetic Oligonucleotide
  source 1..19: mol_type = other DNA
gcttcaatggtccacagtt

SEQ ID NO: 105 - DNA, 19 bp, synthetic construct
  misc_feature 1..19: note = Synthetic Oligonucleotide
  source 1..19: mol_type = other DNA
gcttcaatggtccacagtt

SEQ ID NO: 106 - DNA, 23 bp, synthetic construct
  misc_feature 1..23: note = Synthetic Oligonucleotide
  source 1..23: mol_type = other DNA
  modified_base 12: mod_base = OTHER; note = uracil
gatgatgatcctgcatcactaac

SEQ ID NO: 107 - DNA, 34 bp, synthetic construct
  misc_feature 1..34: note = Synthetic Oligonucleotide
  source 1..34: mol_type = other DNA
cgctgctggcacagatgactggaacatagcagcg

SEQ ID NO: 108 - DNA, 28 bp, synthetic construct
  misc_feature 1..28: note = Synthetic Oligonucleotide
  source 1..28: mol_type = other DNA
cgctgctggcacagatgactggaacata

SEQ ID NO: 109 - DNA, 36 bp, synthetic construct
  misc_feature 1..36: note = Synthetic Oligonucleotide
  source 1..36: mol_type = other DNA
ccgagcaagtctgctggcacagatgactgggctcgg

SEQ ID NO: 110 - DNA, 30 bp, synthetic construct
  misc_feature 1..30: note = Synthetic Oligonucleotide
  source 1..30: mol_type = other DNA
ccgagcaagtctgctggcacagatgactgg

SEQ ID NO: 111 - DNA, 38 bp, synthetic construct
  misc_feature 1..38: note = Synthetic Oligonucleotide
  source 1..38: mol_type = other DNA
ccgagcaagtctgctggcacagatgactggttgctcgg

SEQ ID NO: 112 - DNA, 30 bp, synthetic construct; identical to SEQ ID NO: 110
  misc_feature 1..30: note = Synthetic Oligonucleotide
  source 1..30: mol_type = other DNA

SEQ ID NO: 113 - DNA, 33 bp, synthetic construct
  misc_feature 1..33: note = Synthetic Oligonucleotide
  source 1..33: mol_type = other DNA
cgccagtcatctgtgccagcagacttgctggcg

SEQ ID NO: 114 - DNA, 27 bp, synthetic construct
  misc_feature 1..27: note = Synthetic Oligonucleotide
  source 1..27: mol_type = other DNA
cgccagtcatctgtgccagcagacttg

SEQ ID NO: 115 - DNA, 24 bp, synthetic construct
  misc_feature 1..24: note = Synthetic Oligonucleotide
  source 1..24: mol_type = other DNA
tagtatgttgatgcttgcaagttc

SEQ ID NO: 116 - DNA, 984 bp, unidentified
  source 1..984: mol_type = unassigned DNA; note = Influenza A virus
atgagtcttctaaccgaggtcgaaacgtacgttctttctatcataccgtcaggccccctcaaagccgagatcgcgcagagactggaaagtgtctttgcaggaaagaacacagatcttgaggctctcatggaatggctaaagacaagaccaatcttgtcacctctgactaagggaattttaggatttgtgttcacgctcaccgtgcccagtgagcgaggactgcagcgtagacgctttgtccaaaatgccctgaatgggaatggggacccaaacaacatggatagagcagttaaactatacaagaagctcaaaagagaaataacgttccatggggccaaggaggtgtcactaagctattcaactggtgcacttgccagttgcatgggcctcatatacaacaggatgggaacagtgaccacagaagctgcttttggtctagtgtgtgccacttgtgaacagattgctgattcacagcatcggtctcacagacagatggctacaaccaccaatccactaatcaggcatgagaacagaatggtgctggctagcactacggcaaaggctatggaacagatggctggatcgagtgaacaggcagcggaggccatggaggttgctaatcagactaggcagatggtacatgcaatgagaactattgggactcatcctagctccagtacgggtctgaaagatgaccttcttgaaaatttgcaggcctaccagaagcgaatgggagtgcagatgcagcgattcaagtgatcttctcgccattgcagcaaatatcattgggatcttgcacctgatattgtggattactgatcgtctttttttcaaatgtatttatcgtcgctttaaatacggtttgaaaagagggccttctacggaaggagggcctgagtccatgagggaagaatatcaacaggaacagcagagtgctgtggatgttgacgatggtcattttgtcaacatagagctagagtaaaa

SEQ ID NO: 117 - DNA, 1076 bp, unidentified
  source 1..1076: mol_type = unassigned DNA; note = Influenza B virus
atgtcgctgtttggagacacaattgcctacctgctttcattgacagaagatggagaaggcaaagcagaactagcagaaaaattacactgttggttcggtgggaaagaatttgacctagactctgccttggaatggataaaaaacaaaagatgcttaactgatatacagaaagcactaattggtgcatctatctgctttttaaaacccaaagaccaggaaagaaaaagaagattcatcacagagcccctatcaggaatgggaacaacagcaacaaaaaagaagggcctgattctagctgagagaaaaatgagaaaatgtgtgagcttccatgaagcatttgaaatagcagaaggccatgaaagctcagcgttactgtattgtctcatggtcatgtacctgaatcctggaaattattcaatgcaagtaaaactaggaacgctctgtgctttgtgcgagaaacaagcatcacattcacacagggctcatagcagagcagcgagatcttcagtgcccggagtgagacgagaaatgcagatggtctcagctatgaacacagcaaaaacaatgaatggaatgggaaaaggagaagacgtccaaaaactggcagaagaactgcaaagcaacattggagtattgagatctctgggggcaagccaaaagaatggggaaggaattgcaaaggatgtaatggaagtgctaaagcagagctctatgggaaattcagctcttgtgaagaaatacctataatgctcgaaccatttcagattctttcaatttgttcttttattttatcagctctccatttcatggcctggacaataggacatttgaatcaaataaaaagaggagtaaacatgaaaatacgaataaaggggccaaataaagagacgataaacagagaggtatcaattttgagacacaattaccaaaaagaaattcaggctaaagaagcaatgaaggaagtactctctgacaacatggaggtattgagtgaccacatagtaattgaggggctttctgcagaagagataataaaaatgggtgaaacagttttggaggtagaaaaatcgcattaa

SEQ ID NO: 118 - DNA, 15226 bp, unidentified
  source 1..15226: mol_type = unassigned DNA; note = respiratory syncytial virus
acgcgaaaaaatgcgtacaacaaacttgcgtaaaccaaaaaaatggggcaaataagaatttgataagtaccacttaaatttaactcccttggttagagatgggcagcaattcgttgagtatgataaaagttagattacaaaatttgtttgacaatgatgaagtagcattgttaaaaataacatgctatactgacaaattaatacatttaactaatgctttggctaaggcagtgatacatacaatcaaattgaatggcattgtgtttgtgcatgttattacaagtagtgatatttgccctaataataatattgtagtaaaatccaatttcacaacaatgccagtgctacaaaatggaggttatatatgggaaatgatggaattaacacattgctctcaacctaatggtctaatagatgacaattgtgaaattaaattctccaaaaaactaagtgattcaacaatgaccaattatatgaatcaattatctgaattacttggatttgatcttaatccataaattataattaatatcaactagcaaatcaatgtcactagcaccattagttaatataaaacttaacagaagacaaaaatggggcaaataaatcaactcagccaacccaaccatggacacaacccacaatgataccacaccacaaagactgatgatcacagacatgagaccgttgtcacttgagactacaataacatcactaaccagagacatcataacacacagatttatatacttaataaatcatgaatgcatagtgagaaaacttgatgaaagacaggccacatttacattcctggtcaactatgaaatgaaactattgcacaaagtaggaagcactaaatataaaaaatatactgaatacaacacaaaatatggcactttccctatgccgatattcatcaatcatgatgggttcttagaatgcattggcattaagcctacaaagcatactcccataatatacaagtatgatctcaatccatgaatttcaacacaagattcacacaatccaaaacaacaactttatgcataactacactccatagtccaaatggagcctgaaaattatagtaatttaaaattaaggagagacataagatagaagatggggcaaatacaaagatggctcttagcaaagtcaagttgaatgatacactcaacaaagatcaacttctgtcatctagcaaatacaccatccaacggagcacaggagatagtattgatactcctaattatgatgtgcagaaacacatcaataagttatgtggcatgttattaatcacagaagatgctaatcataaattcactgggttaataggtatgttatatgctatgtctaggttaggaagagaagacaccataaaaatactcagagatgcgggatatcatgtaaaagcaaatggagtagatgtaacaacacatcgtcaagacatcaatgggaaagaaatgaaatttgaagtgttaacattggcaagcttaacaactgaaattcaaatcaacattgagatagaatctagaaaatcctacaaaaaaatgctaaaagaaatgggagaggtagctccagaatacaggcatgattctcctgattgtgggatgataatattatgtatagcagcattagtaataaccaaattggcagcaggggatagatctggtcttacagccgtgattaggagagctaataatgtcctaaaaaatgaaatgaaacgttacaaaggcttactacccaaggatatagccaacagcttctatgaagtgtttgaaaaacatccccactttatagatgtttttgttcattttggtatagcacaatcttccaccagaggtggcagtagagttgaagggatttttgcaggattgtttatgaatgcctatggtgcagggcaagtaatgctacggtggggagtcttagcaaaatcagttaaaaatattatgttaggacatgctagtgtgcaagcagaaatggaacaagttgttgaggtttatgaatatgcccaaaaattgggtggagaagcaggattctaccatatattgaacaacccaaaagcatcattattatctttgactcaatttcctcacttttccagtgtagtattaggcaatgctgctggcctaggcataatgggagagtacagaggtacaccgaggaatcaagatctatatgatgcagcaaaggcatatgctgaacaactcaaagaaaatggtgtgattaactacagtgtattagacttgacagcagaagaactagaggctatcaaacatcagcttaatccaaaagataatgatgtagagctttgagttaataaaaaatggggcaaataaatcatcatggaaaagtttgctcctgaattccatggagaagatgcaaacaacagggctactaaattcctagaatcaataaagggcaaattcacatcacctaaagatcccaagaaaaaagatagtatcatatctgtcaactcaatagatatagaagtaaccaaagaaagccctataacatcaaattcaaccattattaacccaacaaatgagacagatgataatgcagggaacaagcccaattatcaaagaaaacctctagtaagtttcaaagaagaccctataccaagtgataatcccttttcaaaactatacaaagaaaccatagagacatttgataacaatgaagaagaatctagctattcatatgaagaaataaatgatcagacgaacgataatataactgcaagattagataggattgatgaaaaattaagtgaaatactaggaatgcttcacacattagtagtagcaagtgcaggacctacatctgctagggatggtataagagatgccatggttggtttaagagaagaaatgatagaaaaaatcagaactgaagcattaatgaccaatgacagattagaagctatggcaagactcaggaatgaggaaagtgaaaagatggcaaaagacacatcagatgaagtgtctctcaatccaacatcagagaaattgaacaacctgttggaagggaatgatagtgacaatgatctatcacttgaagatttctgattagttacaaatctgcacttcaacacacaacaccaacagaagaccaacaaacaaaccaacccactcatccaaccaaacatccatccgccaatcagccaaacagccaacaaaacaaccagccaatccaaaaccagccacctggaaaaaatcgacaatatagttacaaaaaaagaaaagggtggggcaaatatggaaacatacgtgaacaagcttcacgaaggctccacatacacagctgctgttcaatacaatgtcctagaaaaagacgatgaccctgcatcacttacaatatgggtgcccatgttccaatcatctatgccagcagatttacttataaaagaactagctaatgtcaacatactagtgaaacaaatatccacacccaagggaccttcactaagagtcatgataaactcaagaagtgcattgctagcacaaatgcccagcaaatttaccatatgtgctaatgtgtccttggatgaaagaagcaaactggcatatgatgtaaccacaccctgtgaaatcaaggcatgtagtctaacatgcctaaaatcaaaaaatatgttaactacagttaaagatctcactatgaagacactcaaccccacacatgatattattgctttatgtgaatttgaaaacatagtaacatcaaaaaaagtcataataccaacatacctaagatccatcagtgtcagaaataaagatctgaacacacttgaaaatataacaaccactgaattcaaaaatgccatcacaaatgcaaaaatcatcccttactcaggattactattagtcatcacagtgactgacaacaaaggagcattcaaatacataaagccgcaaagtcaattcatagtagatcttggagcttacctagaaaaagaaagtatatattatgttaccacaaattggaagcacacagctacacgatttgcaatcaaacccatggaagattaacctttttcctccacatcagtgagtcaattcatacaaactttctacctacattcttcacttcaccattacaatcacaaacactctgtggttcaaccaatcaaacaaaacttatctgaagtctcagatcatcccaagtcattgttcatcagatctagtaatcaaataagttaataaaaatatacacatggggcaaataatcatcggaggaaatccaactaatcacaatatctgttaacatagacaagtcaacacaccagacagaatcaaccaatggaaaatacatccataacaatagaattctcaagcaaattctggccttactttacactaatacacatgatcacaacaataatctctttgctaatcataatctccatcatgactgcaatactaaacaaactttgtgaatataacgtattccataacaaaacctttgagttaccaagagctcgagtcaacacatagcattcatcaatctaatagctcaaaatagtaaccttgcatttaaaagtgaacaacccccacctctttacaacacctcattaacatcccaccatgcaaaccaccatccatactataaagtagttaattaaaaatagtcataacaatgaactaggatatcaagactaacaataacgttggggcaaatgcaaacatgtccaaaaacaaggaccaacgcaccgctaagacactagaaaagacctgggacactctcaatcatttattattcatatcatcgggcttatataagttaaatcttaaatctatagcacaaatcacattatccattctggcaatgataatctcaacttcacttataattacagccatcatattcatagcctcggcaaaccacaaagtcacactaacaactgcaatcatacaagatgcaacaagccagatcaagaacacaaccccaacatacctcactcaggatcctcagcttggaatcagcttctccaatctgtctgaaattacatcacaaaccaccaccatactagcttcaacaacaccaggagtcaagtcaaacctgcaacccacaacagtcaagactaaaaacacaacaacaacccaaacacaacccagcaagcccactacaaaacaacgccaaaacaaaccaccaaacaaacccaataatgattttcacttcgaagtgtttaactttgtaccctgcagcatatgcagcaacaatccaacctgctgggctatctgcaaaagaataccaaacaaaaaaccaggaaagaaaaccaccaccaagcctacaaaaaaaccaaccttcaagacaaccaaaaaagatctcaaacctcaaaccactaaaccaaaggaagtacccaccaccaagcccacagaagagccaaccatcaacaccaccaaaacaaacatcacaactacactgctcaccaacaacaccacaggaaatccaaaactcacaagtcaaatggaaaccttccactcaacctcctccgaaggcaatctaagcccttctcaagtctccacaacatccgagcacccatcacaaccctcatctccacccaacacaacacgccagtagttattaaaaaacatattatcacaaaaggccatgaccaactcaaacagaatcaaaataaactctggggcaaataacaatggagttgccaatcctcaaagcaaatgcaattaccacaatcctcgctgcagtcacattttgctttgcttctagtcaaaacatcactgaagaattttatcaatcaacatgcagtgcagttagcaaaggctatcttagtgctctaagaactggttggtatactagtgttataactatagaattaagtaatatcaaggaaaataagtgtaatggaacagatgctaaggtaaaattgataaaccaagaattagataaatataaaaatgctgtaacagaattgcagttgctcatgcaaagcacaacagcagcaaacaatcgagccagaagagaactaccaaggtttatgaattatacactcaacaataccaaaaaaaccaatgtaacattaagcaagaaaaggaaaagaagatttcttggttttttgttaggtgttggatctgcaatcgccagtggcattgctgtatctaaggtcctgcacttagaaggagaagtgaacaagatcaaaagtgctctactatccacaaacaaggccgtagtcagcttatcaaatggagttagtgtcttaaccagcaaagtgttagacctcaaaaactatatagataaacaattgttacctattgtgaataagcaaagctgcagaatatcaaatatagaaactgtgatagagttccaacaaaagaacaacagactactagagattaccagggaatttagtgttaatgcaggtgtaactacacctgtaagcacttacatgttaactaatagtgaattattgtcattaatcaatgatatgcctataacaaatgatcagaaaaagttaatgtccaacaatgttcaaatagttagacagcaaagttactctatcatgtccataataaaagaggaagtcttagcatatgtagtacaattaccactatatggtgtgatagatacaccttgttggaaattacacacatcccctctatgtacaaccaacacaaaagaagggtcaaacatctgtttaacaagaactgacagaggatggtactgtgacaatgcaggatcagtatctttcttcccacaagctgaaacatgtaaagttcaatcgaatcgagtattttgtgacacaatgaacagtttaacattaccaagtgaagtaaatctctgcaatgttgacatattcaatcccaaatatgattgtaaaattatgacttcaaaaacagatgtaagcagctccgttatcacatctctaggagccattgtgtcatgctatggcaaaactaaatgtacagcatccaataaaaatcgtggaatcataaagacattttctaacgggtgtgattatgtatcaaataaaggggtggacactgtgtctgtaggtaacacattatattatgtaaataagcaagaaggcaaaagtctctatgtaaaaggtgaaccaataataaatttctatgacccattagtattcccctctgatgaatttgatgcatcaatatctcaagtcaatgagaagattaaccagagtttagcatttattcgtaaatccgatgaattattacatcatgtaaatgctggtaaatcaaccacaaatatcatgataactactataattatagtgattatagtaatattgttatcattaattgctgttggactgctcctatactgtaaggccagaagcacaccagtcacactaagcaaggatcaactgagtggtataaataatattgcatttagtaactgaataaaaatagcacctaatcatgttcttacaatggtttactatctgctcatagacaacccatctatcattggattttcttaaaatctgaacttcatcgaaactcttatctataaaccatctcacttacactatttaagtagattcctagtttatagttatataaaacacaattgaataccagattaacttactatctgtaaaaatgagaactggggcaaatatgtcacgaaggaatccttgcaaatttgaaattcgaggtcattgcttgaatggtaagagatgtcattttagtcataattattttgaatggccaccccatgcactgctcgtaagacaaaactttatgttaaacagaatacttaagtctatggataaaagtatagataccttatcagaaataagtggagctgcagagttggacagaacagaagagtatgctcttggtgtagttggagtgctagagagttatataggatcaataaataatataactaaacaatcagcatgtgttgccatgagcaaactcctcactgaactcaatagtgatgatatcaaaaaactgagagacaatgaagagctaaattcacccaagataagagtgtacaatactgtcatatcatatattgaaagcaacaggaaaaacaataaacaaactatccatctgttaaaaagattgccagcagacgtattgaagaaaaccatcaaaaacacattggatatccacaagagcataaccatcaacaacccaaaagaattaactgttagtgatacaaatgaccatgccaaaaataatgatactacctgacaaatatccttgtagtataacttccatactaataacaagtagatgtagagtcactatgtataatcgaaagaacacactatatttcaatcaaaacaacccaaataaccatatgtactcaccgaatcaaacattcaatgaaatccattggacctcacaagacttgattgacacaattcaaaattttctacagcatctaggtgttattgaggatatatatacaatatatatattagtgtcataacactcaatcctaatactgaccatatcgttgaattattaattcaaataattcaagctgtgggacaaaatggatcccattattaatggaaattctgctaatgtttatctaaccgatagttatttaaaaggtgttatctctttctcagagtgtaatgctttaggaagttacatattcaatggtccttatctcaaaaatgattataccaacttaattagtagacaaaatccattaatagaacacatgaatctaaagaaactaaatataacacagtccttaatatctaagtatcataaaggtgaaataaaattagaagagcctacttattttcagtcattacttatgacatacaagagtatgacctcgttggaacagattgctaccactaatttacttaaaaagataataagaagagctatagaaataagtgatgtcaaagtctatgctatattgaataaactagggcttaaagaaaaggacaagattaaatccaacaatggacaggatgaagacaactcagttattacgaccataatcaaagatgatatactttcagctgttaaggataatcaatctcatcttaaagcagacaaaaatcactctacaaaacaaaaagacacaatcaaaacaacactcttgaagaaattaatgtgttcaatgcagcatcctccatcatggttaatacattggtttaatttatacacaaaattaaacaacatattaacacagtatcgatcaaatgaggttaaaaaccatgggtttatattgatagataatcaaactcttagtggatttcaatttattttgaatcaatatggttgtatagtttatcataaggaactcaaaagaattactgtgacaacctataatcaattcttgacatggaaagatattagccttagtagattaaatgtttgtttaattacatggattagtaactgcttgaacacattaaataaaagcttaggcttaagatgcggattcaataatgttatcttgacacaactattcctttatggtgattgtatactaaagctatttcacaatgaggggttctacataataaaagaggtagagggatttattatgtctctaattttaaatataacagaagaagatcaattcagaaaacgattttataatagtatgctcaacaacatcacagatgctgctaataaagctcagaaaaatctgctatcaagagtatgtcatacattattagataagacagtatccgataatataataaatggcagatggataattctattaagtaagttccttaaattaattaagcttgcaggtgacaataaccttaacaatctgagtgaactatattttttgttcagaatatttggacacccaatggtagatgaaagacaagccatggatgctgttaaagttaattgcaatgagaccaaattttacttgttaagcagtttgagtatgttaagaggtgcctttatatatagaattataaaagggtttgtaaataattacaacagatggcctactttaagaaatgctattgttttacccttaagatggttaacttactataaactaaacacttatccttctttgttggaacttacagaaagagatttgattgtgttatcaggactacgtttctatcgtgagtttcggttgcctaaaaaagtggatcttgaaatgattataaatgataaagctatatcaccccctaaaaatttgatatggactagtttccctagaaattatatgccgtcacacatacaaaactatatagaacatgaaaaattaaaattttccgagagtgataaatcaagaagagtattagagtattatttaagagataacaaattcaatgaatgtgatttatacaactgtgtagttaatcaaagttatctcaacaaccctaatcatgtggtatcattgacaggcaaagaaagagaactcagtgtaggtagaatgtttgcaatgcaaccgggaatgttcagacaggttcaaatattggcagagaaaatgatagctgaaaacattttacaattctttcctgaaagtcttacaagatatggtgatctagaactacaaaaaatattagaattgaaagcaggaataagtaacaaatcaaatcgctacaatgataattacaacaattacattagtaagtgctctatcatcacagatctcagcaaattcaatcaagcatttcgatatgaaacgtcatgtatttgtagtgatgtgctggatgaactgcatggtgtacaatctctattttcctggttacatttaactattcctcatgtcacaataatatgcacatataggcatgcacccccctatataagagatcatattgtagatcttaacaatgtagatgaacaaagtggattatatagatatcacatgggtggtattgaagggtggtgtcaaaaactatggaccatagaagctatatcactattggatctaatatctctcaaagggaaattctcaattactgctttaattaatggtgacaatcaatcaatagatataagcaaaccagtcagactcatggaaggtcaaactcatgctcaagcagattatttgctagcattaaatagccttaaattactgtataaagagtatgcaggcataggtcacaaattaaaaggaactgagacttatatatcacgagatatgcaatttatgagtaaaacaattcaacataacggtgtatattaccctgctagtataaagaaagtcctaagagtgggaccgtggataaacactatacttgatgatttcaaagtgagtctagaatctataggtagtttgacacaagaattagaatatagaggtgaaagtctattatgcagtttaatatttagaaatgtatggttatataatcaaattgctctacaattaaaaaatcatgcgttatgtaacaataaattatatttggacatattaaaggttctgaaacacttaaaaaccttttttaatcttgataatattgatacagcattaacattgtatatgaatttacccatgttatttggtggtggtgatcccaacttgttatatcgaagtttctatagaagaactcctgatttcctcacagaggctatagttcactctgtgttcatacttagttattatacaaaccatgacttaaaagataaacttcaagatttgtcagatgatagattgaataagttcttaacatgcataatcacgtttgacaaaaaccctaatgctgaattcgtaacattgatgagagatcctcaagctttagggtctgagagacaagctaaaattactagtgaaatcaatagactggcagttacagaggttttgagtacagctccaaacaaaatattctccaaaagtgcacaacattataccactacagagatagatctaaatgatattatgcaaaatatagaacctacatatcctcacgggctaagagttgtttatgaaagtttacccttttataaagcagagaaaatagtaaatcttatatcaggtacaaaatctataactaacatactggaaaagacttctgccatagacttaacagatattgatagagccactgagatgatgaggaaaaacataactttgcttataaggatacttccattggattgtaacagagataaaagagaaatattgagtatggaaaacctaagtattactgaattaagcaaatatgttagggaaagatcttggtctttatccaatatagttggtgttacatcacccagtatcatgtatacaatggacatcaaatatacaacaagcactatagctagtggcataattatagagaaatataatgttaacagtttaacacgtggtgagagaggaccaactaaaccatgggttggttcatctacacaagagaaaaaaacaatgccagtttataatagacaagttttaaccaaaaaacaaagagatcaaatagatctattagcaaaattggattgggtgtatgcatctatagataacaaggatgaattcatggaagaactcagcataggaacccttgggttaacatatgaaaaggccaaaaaattatttccacaatatttaagtgtcaactatttgcatcgccttacagtcagtagtagaccatgtgaattccctgcatcaataccagcttatagaacaacaaattatcactttgacactagccctattaatcgcatattaacagaaaagtatggtgatgaagatattgacatagtattccaaaactgtataagctttggccttagcttaatgtcagtagtagaacaatttactaatgtatgtcctaacagaattattctcatacctaagcttaatgagatacatttgatgaaacctcccatattcacaggtgatgttgatattcacaagttaaaacaagtgatacaaaaacagcatatgtttttaccagacaaaataagtttgactcaatatgtggaattattcttaagtaacaaaacactcaaatctggatctcatgttaattctaatttaatattggcacataaaatatctgactattttcataatacttacattttaagtactaatttagctggacattggattctaattatacaacttatgaaagattctaaaggtatttttgaaaaagattggggagagggatatataactgatcatatgtttattaatttgaaagttttcttcaatgcttataagacctatctcttgtgttttcataaaggttatggcaaagcaaaactggagtgtgatatgaacacttcagatcttctatgtgtattggaattaatagacagtagttattggaagtctatgtctaaggtatttttagaacaaaaagttatcaaatacattcttagccaagatgcaagtttacatagagtaaaaggatgtcatagcttcaaattatggtttcttaaacgtcttaatgtagcagaatttacagtttgcccttgggttgttaacatagattatcatccaacacatatgaaagcaatattaacttatatagatcttgttagaatgggattgataaatatagatagaatacacattaaaaataaacacaaattcaatgatgaattttatacttctaatctcttttacattaattataacttctcagataatactcatctattaactaaacatataaggattgctaattcagaattagaaaataattacaacaaattatatcatcctacaccagaaaccctagagaatatactagccaatccgattaaaagtaatgacaaaaagacactgaacgactattgtataggtaaaaatgttgactcaataatgttaccattgttatctaataagaagcttgttaaatcgtctgcaatgattagaaccaattacagcaaacaagacctgtacaatctattccctacggttgtgatcgatagaattatagatcattcaggtaatacagccaaatccaaccaactttacactactacttcccatcaaatatctttagtgcacaatagcacatcactttattgcatgcttccttggcatcatattaatagattcaattttgtatttagttctacaggttgtaaaattagtatagagtatattttaaaagaccttaaaattaaagatcctaattgtatagcattcataggtgaaggagcagggaatttattattgcgtacagtggtggaacttcatcctgacataagatatatttacagaagtctgaaagattgcaatgatcatagtttacctattgagtttttaaggctatacaatggacatatcaacattgattatggtgaaaatttgaccattcctgctacagatgcaaccaacaacattcattggtcttatttacatataaagtttgctgaacctatcagtctttttgtatgtgatgccgaattgcctgtaacagtcaactggagtaaaattataatagaatggagcaagcatgtaagaaaatgcaagtactgttcctcagttaataaatgtacgttaatagtaaaatatcatgctcaagatgatattgatttcaaattagacaatataactatattaaaaacttatgtatgcttaggcagtaagttaaagggatcggaggtttacttagtccttacaataggtcctgcaaatatatttccagtatttaatgtagtacaaaatgctaaattgatactatcaagaaccaaaaatttcatcatgcctaagaaagctgataaagagtctattgatgcaaatattaaaagtttgataccctttctttgttaccctataacaaaaaaaggaattaatactgcattgtcaaaactaaagagtgttgttagtggagatatactatcatattctatagctggacggaatgaagttttcagcaataaacttataaatcataagcatatgaacatcttaaagtggttcaatcatgttttaaatttcagatcaacagaactaaactataaccatttatatatggtagaatctacatatccttacctaagtgaattgttaaacagcttgacaactaatgaacttaaaaaactgattaaaatcacaggtagtctgttatacaactttcataatgaataatgaataaagatcttataataaaaattcctatagctatacactagcactgtattcaattatagttattaaaaaattaaaaatcatataattttttataaaaataacttttagtgaactaatcctaaagttatcattttgatctaggaggaataaatttaaatcccaatctaattggtttatatgtgtattaactaaactacgagatattagtttttgacactttttttctcgt

SEQ ID NO: 119 - DNA, 15225 bp, unidentified
  source 1..15225: mol_type = unassigned DNA; note = respiratory syncytial virus
acgcgaaaaaatgcgtactacaaacttgcacattcggaaaaaatggggcaaataagaatttgataagtgctatttaagtctaaccttttcaatcagaaatggggtgcaattcactgagcatgataaaggttagattacaaaatttatttgacaatgacgaagtagcattgttaaaaataacatgttatactgacaaattaattcttctgaccaatgcattagccaaagcagcaatacatacaattaaattaaacggtatagtttttatacatgttataacaagcagtgaagtgtgccctgataacaacattgtagtaaaatctaactttacaacaatgccaatattacaaaacggaggatacatatgggaattgattgagttgacacactgctctcaattaaacggtctaatggatgataattgtgaaatcaaattttctaaaagactaagtgactcagtaatgactaattatatgaatcaaatatctgatttacttgggcttgatctcaattcatgaattatgtttagtctaactcaatagacatgtgtttattaccattttagttaatataaaaactcatcaaagggaaatggggcaaataaactcacctaatcaatcaaactatgagcactacaaatgacaacactactatgcaaagattaatgatcacggacatgagacccctgtcgatggattcaataataacatctctcaccaaagaaatcatcacacacaaattcatatacttgataaacaatgaatgtattgtaagaaaacttgatgaaagacaagctacatttacattcttagtcaattatgagatgaagctactgcacaaagtagggagtaccaaatacaagaaatacactgaatataatacaaaatatggcactttccccatgcctatatttatcaatcatggcgggtttctagaatgtattggcattaagcctacaaaacacactcctataatatacaaatatgacctcaacccgtaaattccaacaaaaaaaaccaacccaaccaaaccaagctattcctcaaacaacaatgctcaatagttaagaaggagctaatccgttttagtaattaaaaataaaagtaaagccaataacataaattggggcaaatacaaagatggctcttagcaaagtcaagttaaatgatacattaaataaggatcagctgctgtcatccagcaaatacactattcaacgtagtacaggagataatattgacactcccaattatgatgtgcaaaaacacctaaacaaactatgtggtatgctattaatcactgaagatgcaaatcataaattcacaggattaataggtatgttatatgctatgtccaggttaggaagggaagacactataaagatacttaaagatgctggatatcatgttaaagctaatggagtagatataacaacatatcgtcaagatataaatggaaaggaaatgaaattcgaagtattaacattatcaagcttgacatcagaaatacaagtcaatattgagatagaatctagaaaatcctacaaaaaaatgctaaaagagatgggagaagtggctccagaatataggcatgattctccagactgtgggatgataatactgtgtatagcagcacttgtaataaccaaattagcagcaggagacagatcaggtcttacagcagtaattaggagggcaaacaatgtcttaaaaaatgaaataaaacgctacaagggtctcataccaaaggatatagctaacagtttttatgaagtgtttgaaaaacaccctcatcttatagatgtttttgtgcactttggcattgcacaatcatcaacaagagggggtagtagagttgaaggaatctttgcaggattgtttatgaatgcctatggttcagggcaagtaatgctaagatggggagttttagccaaatctgtaaaaaatatcatgctaggtcatgctagtgtccaggcagaaatggagcaagttgtggaagtctatgagtatgcacagaagttgggaggagaagctggattctaccatatattgaacaatccaaaagcatcattgctgtcattaactcaatttcctaacttctcaagtgtggtcctaggcaatgcagcaggtctaggcataatgggagagtatagaggtacgccaagaaaccaggatctttatgatgcagccaaagcatatgcagagcaactcaaagaaaatggagtaataaactacagtgtattagacttaacagcagaagaattggaagccataaagaatcaactcaaccctaaagaagatgatgtagagctttaagttaacaaaaaatacggggcaaataagtcaacatggagaagtttgcacctgaatttcatggagaagatgcaaataacaaagctaccaaattcctagaatcaataaagggcaagttcgcatcatccaaagatcctaagaagaaagatagcataatatctgttaactcaatagatatagaagtaaccaaagagagcccgataacatctggcaccaacatcatcaatccaacaagtgaagccgacagtaccccagaaaccaaagccaactacccaagaaaacccctagtaagcttcaaagaagatctcaccccaagtgacaaccctttttctaagttgtacaaagaaacaatagaaacatttgataacaatgaagaagaatctagctactcatatgaagagataaatgatcaaacaaatgacaacattacagcaagactagatagaattgatgaaaaattaagtgaaatattaggaatgctccatacattagtagttgcaagtgcaggacccacttcagctcgcgatggaataagagatgctatggttggtctgagagaagaaatgatagaaaaaataagagcggaagcattaatgaccaatgataggttagaggctatggcaagacttaggaatgaggaaagcgaaaaaatggcaaaagacacctcagatgaagtgcctcttaatccaacttccaaaaaattgagtgacttgttggaagacaacgatagtgacaatgatctgtcacttgatgatttttgatcagtgatcaactcactcagcaatcaacaacatcaataaaacagacatcaatccattgaatcaactgccagaccgaacaaacaaatgtccgtcagcggaaccaccaaccaatcaatcaaccaactgatccatcagcaacctgacgaaattaacaatatagtaacaaaaaaagaacaagatggggcaaatatggaaacatacgtgaacaagcttcacgaaggctccacatacacagcagctgttcagtacaatgttctagaaaaagatgatgatcctgcatcactaacaatatgggtgcctatgttccagtcatctgtaccagcagacttgctcataaaagaacttgcaagcatcaacatactagtgaagcagatctctacgcccaaaggaccttcactacgagtcacgattaactcaagaagtgctgtgctggctcaaatgcctagtaatttcatcataagcgcaaatgtatcattagatgaaagaagcaaattagcatatgatgtaactacaccttgtgaaatcaaagcatgcagtctaacatgcttaaaagtgaaaagtatgttaactacagtcaaagatcttaccatgaagacattcaaccccactcatgagatcattgctctatgtgaatttgaaaatattatgacatcaaaaagagtaataataccaacctatctaagaccaattagtgtcaaaaacaaggatctgaactcactagaaaacatagcaaccaccgaattcaaaaatgctatcaccaatgcgaaaattattccctatgctggattagtattagttatcacagttactgacaataaaggagcattcaaatatatcaagccacagagtcaatttatagtagatcttggtgcctacctagaaaaagagagcatatattatgtgactactaattggaagcatacagctacacgtttttcaatcaaaccactagaggattaaatttaattatcaacactgaatgacaggtccacatatatcctcaaactacacactatatccaaacatcatgaacatctacactacacacttcatcacacaaaccaatcccactcaaaatccaaaatcactaccagccactatctgctagacctagagtgcgaataggtaaataaaaccaaaatatggggtaaatagacattagttagagttcaatcaatctcaacaaccatttataccgccaattcaatacatatactataaatcttaaaatgggaaatacatccatcacaatagaattcacaagcaaattttggccctattttacactaatacatatgatcttaactctaatctctttactaattataatcactattatgattgcaatactaaataagctaagtgaacataaaacattctgtaacaatactcttgaactaggacagatgcatcaaatcaacacatagtgctctaccatcatgctgtgtcaaattataatcctgtatatataaacaaacaaatccaatcttctcacagagtcatggtgtcgcaaaaccacgccaactatcatggtagcatagagtagttatttaaaaattaacataatgatgaattattagtatgggatcaaaaacaacattggggcaaatgcaaccatgtccaaacacaagaatcaacgcactgccaggactctagaaaagacctgggatactctcaatcatctaattgtaatatcctcttgtttatacagattaaatttaaaatctatagcacaaatagcactatcagttctggcaatgataatctcaacctctctcataattgcagccataatattcatcatctctgccaatcacaaagttacactaacaacggtcacagttcaaacaataaaaaaccacactgaaaaaaacatcaccacctaccttactcaagtcccaccagaaagggttagctcatccaaacaacctacaaccacatcaccaatccacacaaattcagccacaacatcacccaacacaaagtcagaaacacaccacacaacagcacaaaccaaaggcagaaccaccacctcaacacagaccaacaagccgagcacaaaaccacgcctaaaaaatccaccaaaaaaaccaaaagatgattaccattttgaagtgttcaacttcgttccctgtagtatatgtggcaacaatcaactttgcaaatccatctgtaaaacaataccaagcaacaaaccaaagaagaaaccaaccatcaaacccacaaacaaaccaaccaccaaaaccacaaacaaaagagacccaaaaacaccagccaaaacgacgaaaaaagaaactaccaccaacccaacaaaaaaaccaaccctcacgaccacagaaagagacaccagcacctcacaatccactgtgctcgacacaaccacattagaacacacaatccaacagcaatccctccactcaaccacccccgaaaacacacccaactccacacaaacacccacagcatccgagccctctacatcaaattccacccaaaatacccaatcacatgcttagttattcaaaaactacatcttagcagaaaaccgtgacctatcaagcaagaacgaaattaaacctggggcaaataaccatggagctgctgatccacaggttaagtgcaatcttcctaactcttgctattaatgcattgtacctcacctcaagtcagaacataactgaggagttttaccaatcgacatgtagtgcagttagcagaggttattttagtgctttaagaacaggttggtataccagtgtcataacaatagaattaagtaatataaaagaaaccaaatgcaatggaactgacactaaagtaaaacttataaaacaagaattagataagtataagaatgcagtgacagaattacagctacttatgcaaaacacaccagctgccaacaaccgggccagaagagaagcaccacagtatatgaactatacaatcaataccactaaaaacctaaatgtatcaataagcaagaagaggaaacgaagatttctgggcttcttgttaggtgtaggatctgcaatagcaagtggtatagctgtatccaaagttctacaccttgaaggagaagtgaacaagatcaaaaatgctttgttatctacaaacaaagctgtagtcagtctatcaaatggggtcagtgttttaaccagcaaagtgttagatctcaagaattacataaataaccaattattacccatagtaaatcaacagagctgtcgcatctccaacattgaaacagttatagaattccagcagaagaacagcagattgttggaaatcaacagagaattcagtgtcaatgcaggtgtaacaacacctttaagcacttacatgttaacaaacagtgagttactatcattgatcaatgatatgcctataacaaatgatcagaaaaaattaatgtcaagcaatgttcagatagtaaggcaacaaagttattctatcatgtctataataaaggaagaagtccttgcatatgttgtacagctacctatctatggtgtaatagatacaccttgctggaaattacacacatcacctctatgcaccaccaacatcaaagaaggatcaaatatttgtttaacaaggactgatagaggatggtattgtgataatgcaggatcagtatccttctttccacaggctgacacttgtaaagtacagtccaatcgagtattttgtgacactatgaacagtttgacattaccaagtgaagtcagcctttgtaacactgacatattcaattccaagtatgactgcaaaattatgacatcaaaaacagacataagcagctcagtaattacttctcttggagctatagtgtcatgctatggtaaaactaaatgcactgcatccaacaaaaatcgtgggattataaagacattttctaatggttgtgactatgtgtcaaacaaaggagtagatactgtgtcagtgggcaacactttatactatgtaaacaagctggaaggcaagaacctttatgtaaaaggggaacctataataaattactatgaccctctagtgtttccttctgatgagtttgatgcatcaatatctcaagtcaatgaaaaaatcaatcaaagtttagcttttattcgtagatctgatgaattactacataatgtaaatactggcaaatctactacaaatattatgataactacaattattatagtaatcattgtagtattgttatcattaatagctattggtttgctgttgtattgcaaagccaaaaacacaccagttacactaagcaaagaccaactaagtggaatcaataatattgcattcagcaaatagacaaaaaaccacctgatcatgtttcaacaacagtctgctgatcaccaatcccaaatcaacccataacaaacacttcaacatcacagtacaggctgaatcatttcttcacatcatgctacccacacaactaagctagatccttaactcatagttacataaaaacctcaagtatcacaatcaaacactaaatcaacacatcattcacaaaattaacagctggggcaaatatgtcgcgaagaaatccttgtaaatttgagattagaggtcattgcttgaatggtagaagatgtcactacagtcataattactttgaatggcctcctcatgccttactagtgaggcaaaacttcatgttaaacaagatactcaagtcaatggacaaaagcatagacactttgtctgaaataagtggagctgctgaactggacagaacagaagaatatgctcttggtatagttggagtgctagagagttacataggatctataaacaacataacaaaacaatcagcatgtgttgctatgagtaaacttcttattgagatcaatagtgatgacattaaaaagctgagagataatgaagaacccaattcacctaagataagagtgtacaatactgttatatcatacattgagagcaatagaaaaaacaacaagcaaacaatccatctgctcaaaagactaccagcagacgtgctgaagaagacaataaaaaacacattagatatccacaaaagcataatcataagcaacccaaaagagtcaaccgtgaatgatcaaaatgaccaaaccaaaaataatgatattaccggataaatatccttgtagtatatcatccatattgatttcaagtgaaagcatgattgctacattcaatcataaaaacatattacaatttaaccataaccatttggataaccaccagcgtttattaaataatatatttgatgaaattcattggacacctaaaaacttattagatgccactcaacaatttctccaacatcttaacatccctgaagatatatatacaatatatatattagtgtcataatgcttggccataacgattctatatcatccaaccataaaactatcttaataaggttatgggacaaaatggatcccattattaatggaaactctgctaatgtgtatctaactgatagttatttaaaaggtgttatctctttttcagaatgtaatgctttagggagttacctttttaacggcccttatctcaaaaatgattacaccaacttaattagtagacaaagtccactactagagcatatgaatcttaaaaaactaactataacacagtcattaatatctagatatcataaaggtgaactgaaattagaagaaccaacttatttccagtcattacttatgacatataaaagcatgtcctcgtctgaacaaattgctacaactaacttacttaaaaaaataatacgaagagctatagaaataagtgatgtaaaggtgtacgccatcttgaataaactaggactaaaggaaaaggacagagttaagcccaacaataattcaggtgatgaaaactcagtacttacaactataattaaagatgatatactttcggctgtggaaagcaatcaatcatatacaaattcagacaaaaatcactcagtaaatcaaaatatcactatcaaaacaacactcttgaaaaaattgatgtgttcaatgcaacatcctccatcatggttaatacactggttcaatttatatacaaaattaaataacatattaacacaatatcgatcaaatgaggtaaaaagtcatgggtttatattaatagataatcaaactttaagtggttttcagtttattttaaatcaatatggttgtatcgtttatcataaaggactcaaaaaaatcacaactactacttacaatcaatttttaacatggaaagacatcagccttagcagattaaatgtttgcttaattacttggataagtaattgtttgaatacattaaataaaagcttagggctgagatgtggattcaataatgttgtgttatcacaattatttctttatggagattgtatactgaaattatttcataatgaaggcttctacataataaaagaagtagagggatttattatgtctttaattctaaacataacagaagaagatcaatttaggaaacgattttataatagcatgctaaataacatcacagatgcagctattaaggctcaaaagaacctactatcaagggtatgtcacactttattagacaagacagtgtctgataatatcataaatggtaaatggataatcctattaagtaaatttcttaaattgattaagcttgcaggtgataataatctcaataatttgagtgagctatattttctcttcagaatctttggacatccaatggttgatgaaagacaagcaatggatgctgtaagaattaactgtaatgaaactaagttctacttattaagtagtctaagtacgttaagaggtgctttcatttatagaatcataaaagggtttgtaaatacctacaacagatggcccactttaaggaatgctattgtcctacctctaagatggttaaactattataaacttaatacttatccatctctacttgaaatcacagaaaatgatttgattattttatcaggattgcggttctatcgtgaatttcatctgcctaaaaaagtggatcttgaaatgataataaatgacaaagccatttcacctccaaaagatctaatatggactagttttcctagaaattacatgccatcacatatacaaaattatatagaacatgaaaagttgaagttctctgaaagcgacagatcaagaagagtactagagtattacttgagagataataaattcaatgaatgcgatctatacaattgtgtagtcaatcaaagctatctcaacaactctaatcacgtggtatcactaactggtaaagaaagagagctcagtgtaggtagaatgtttgctatgcaaccaggtatgtttaggcaaatccaaatcttagcagagaaaatgatagccgaaaatattttacaattcttccctgagagtttgacaagatatggtgatctagagcttcaaaagatattagaattaaaagcaggaataagcaacaagtcaaatcgttataatgataactacaacaattatatcagtaaatgttctatcattacagatcttagcaaattcaatcaagcatttagatatgaaacatcatgtatctgcagtgatgtattagatgaactgcatggagtacaatctctgttctcttggttgcatttaacaatacctcttgtcacaataatatgtacatatagacatgcacctcctttcataaaggatcatgttgttaatcttaatgaagttgatgaacaaagtggattatacagatatcatatgggtggtattgagggctggtgtcaaaaactgtggaccattgaagctatatcattattagatctaatatctctcaaagggaaattctctatcacagctctgataaatggtgataatcagtcaattgatataagtaaaccagttagacttatagagggtcagacccatgctcaagcagattatttgttagcattaaatagccttaaattgctatataaagagtatgcaggtataggccataagcttaagggaacagagacctatatatcccgagatatgcagttcatgagcaaaacaatccagcacaatggagtgtactatccagccagtatcaaaaaagtcctgagagtaggtccatggataaatacaatacttgatgattttaaagttagtttagaatctataggtagcttaacacaggagttagaatacagaggggaaagcttattatgcagtttaatatttaggaacatttggttatacaatcaaattgctttgcaactccgaaatcatgcattatgtaacaataagctatatttagatatattgaaagtattaaaacacttaaaaactttttttaatcttgatagtatcgatatggcgttatcattgtatatgaatttgcctatgctgtttggtggtggtgatcctaatttgttatatcgaagcttttataggagaactccagacttccttacagaagctatagtacattcagtgtttgtgttgagctattatactggtcacgatttacaagataagctccaggatcttccagatgatagactgaacaaattcttgacatgtgtcatcacattcgataaaaatcccaatgccgagtttgtaacattgatgagggatccacaggcgttagggtctgaaaggcaagctaaaattactagtgagattaatagattagcagtaacagaagtcttaagtatagctccaaacaaaatattttctaaaagtgcacaacattatactaccactgagattgatctaaatgacattatgcaaaatatagaaccaacttaccctcatggattaagagttgtttatgaaagtctacctttttataaagcagaaaaaatagttaatcttatatcaggaacaaaatccataactaatatacttgaaaaaacatcagcaatagatacaactgatattaatagggctactgatatgatgaggaaaaatataactttacttataaggatacttccactagattgtaacaaagacaaaagagagttattaagtttagaaaatcttagtataactgaattaagcaagtatgtaagagaaagatcttggtcattatccaatatagtaggagtaacatcgccaagtattatgttcacaatggacattaaatatacaactagcactatagccagtggtataattatagaaaaatataatgttaatagtttaactcgtggtgaaagaggacctactaagccatgggtaggttcatctacgcaggagaaaaaaacaatgccagtgtacaatagacaagttttaaccaaaaagcaaagagaccaaatagatttattagcaaaattagactgggtatatgcatccatagacaacaaagatgaattcatggaagaactgagtactggaacacttggactgtcatatgaaaaagccaaaaagttgtttccacaatatctaagtgtcaattatttacaccgtttaacagtcagtagtagaccatgtgaattccctgcatcaataccagcttatagaacaacaaattatcatttcgatactagtcctatcaatcatgtattaacagaaaagtatggagatgaagatatcgacattgtgtttcaaaattgcataagttttggtcttagcctgatgtcggttgtggaacaattcacaaacatatgtcctaatagaattattctcataccgaagctgaatgagatacatttgatgaaacctcctatatttacaggagatgttgatatcatcaagttgaagcaagtgatacaaaaacagcatatgttcctaccagataaaataagtttaacccaatatgtagaattattcctaagtaacaaagcacttaaatctggatctaacatcaattctaatttaatattagtacataaaatgtctgattattttcataatgcttatattttaagtactaatttagctggacattggattctaattattcaacttatgaaagattcaaaaggtatttttgaaaaagattggggagaggggtacataactgatcatatgttcattaatttgaatgttttctttaatgcttataagacttatttgctatgttttcataaaggttatggtaaagcaaaattagaatgtgatatgaacacttcagatcttctttgtgttttggagttaatagacagtagctactggaaatctatgtctaaagttttcctagaacaaaaagtcataaaatacatagtcaatcaagacacaagtttgcatagaataaaaggctgtcacagttttaagttgtggtttttaaaacgccttaataatgctaaatttaccgtatgcccttgggttgttaacatagattatcacccaacacatatgaaagctatattatcttacatagatttagttagaatggggttaataaatgtagataaattaaccattaaaaataaaaacaaattcaatgatgaattttacacatcaaatctcttttacattagttataacttttcagacaacactcatttgctaacaaaacaaataagaattgctaattcagaattagaagataattataacaaactatatcacccaaccccagaaactttagaaaatatatcattaattcctgttaaaagtaataatagtaacaaacctaaattttgtataagtggaaataccgaatctataatgatgtcaacattctctaataaaatgcatattaaatcttccactgttaccacaagattcaattatagcaaacaagacttgtacaatttatttccaaatgttgtgatagacaggattatagatcattcaggtaatacagcaaaatctaaccaactttacatcaccacttcacatcagacatctttagtaaggaatagtgcatcactttattgcatgcttccttggcatcatgtcaatagatttaactttgtatttagttccacaggatgcaagatcagtatagagtatattttaaaagatcttaagattaaggaccccagttgtatagcattcataggtgaaggagctggtaacttattattacgtacggtagtagaacttcatccagacataagatacatttacagaagtttaaaagattgcaatgatcatagtttacctattgaatttctaagattatacaacgggcatataaacatagattatggtgagaatttaaccattcctgctacagatgcaactaataacattcattggtcttatttacatataaaatttgcagaacctattagcatctttgtctgcgatgctgaattacctgttacagccaattggagtaaaattataattgaatggagtaagcatgtaagaaagtgcaagtactgttcttctgtaaatagatgcattttaatcgcaaaatatcatgctcaagatgatattgatttcaaattagataacattactatattaaaaacttacgtgtgcctaggtagcaagttaaaaggatctgaagtttacttagtccttacaataggccctgcaaatatacttcctgtttttgatgttgtgcaaaatgctaaattgattttttcaagaactaaaaatttcattatgcctaaaaaaactgacaaggaatctatcgatgcaaatattaaaagcttaatacctttcctttgttaccctataacaaaaaaaggaattaagacttcattgtcaaaattgaagagtgtagttaatggggatatattatcatattctatagctggacgtaatgaagtattcagcaacaagcttataaaccacaagcatatgaatatcctaaaatggctagatcatgttttaaattttagatcagctgaacttaattacaatcatttatacatgatagagtccacatatccttacttaagtgaattgttaaatagtttaacaaccaatgagctcaagaaactgattaaaataacaggtagtgtactatacaaccttcccaacgaacagtaacttaaaatatcattaacaagtttggtcaaatttagatgctaacacatcattatattatagttattaaaaaatatgcaaacttttcaataatttagcttactgattccaaaattatcattttatttttaaggggttgaataaaagtctaaaactaacaatgatacatgtgcatttacaacacaacgagacattagtttttgacactttttttctcgt